European Patent Specification EP 3 087 082 B1, published October 11, 2023. Title: ATP synthase inhibitors and steroid alkaloids and uses thereof as antimicrobial agents and as potentiators for aminoglycosides against pathogenic bacteria. Applicant: SOCPRA - Sciences et Génie s.e.c. MARSAULT, Eric MALOUIN, François CHAGNON, Félix GUAY, Isabelle BOULANGER, Simon. Application N.A.. The sequence listing filed with the application follows.

SEQUENCE LISTING (36 sequences)

SEQ ID NO: 1 - DNA, 11 bp, Staphylococcus aureus
taggagcaggt

SEQ ID NO: 2 - DNA, 11 bp, Staphylococcus aureus
taggatcaggt

SEQ ID NO: 3 - DNA, 11 bp, Staphylococcus aureus
aattgcattca

SEQ ID NO: 4 - DNA, 11 bp, Staphylococcus aureus
aattacattca

SEQ ID NO: 5 - protein, 70 aa, Staphylococcus aureus
MNLIAAAIAIGLSALGAGIGNGLIVSRTVEGVARQPEARGQLMGIMFIGVGLVEALPIIGVVIAFMTFAG

SEQ ID NO: 6 - protein, 72 aa, Listeria monocytogenes
MSLGVIAAAIAVGLGALGAGIGNGLIVSKTVEGVARQPEARSMLQTIMFIGIGLVEALPIIAVVIAFMVLNK

SEQ ID NO: 7 - protein, 70 aa, Bacillus subtilis
MNLIAAAIAIGLGALGAGIGNGLIVSRTVEGIARQPEAGKELRTLMFMGIALVEALPIIAVVIAFLAFFG

SEQ ID NO: 8 - protein, 72 aa, Bacillus cereus
MSLGVIAAAIAIGLSALGAGIGNGLIVSRTIEGVARQPELKGALQTIMFIGVALVEALPIIGVVIAFIVMNK

SEQ ID NO: 9 - protein, 72 aa, Bacillus anthracis; identical to SEQ ID NO: 8

SEQ ID NO: 10 - protein, 66 aa, Streptococcus pneumoniae
MNLTFLGLCIACMGVSVGEGLLMNGLFKSVARQPDMLSEFRSLMFLGVAFIEGTFFVTLVFSFIIK

SEQ ID NO: 11 - protein, 79 aa, Escherichia coli
MENLNMDLLYMAAAVMMGLAAIGAAIGIGILGGKFLEGAARQPDLIPLLRTQFFIVMGLVDAIPMIAVGLGLYVMFAVA

SEQ ID NO: 12 - protein, 86 aa, Mycobacterium smegmatis
MDLDPNAIITAGALIGGGLIMGGGAIGAGIGDGIAGNALISGIARQPEAQGRLFTPFFITVGLVEAAYFINLAFMALFVFATPGLQ

SEQ ID NO: 13 - protein, 142 aa, Homo sapiens
MFACAKLACTPSLIRAGSRVAYRPISASVLSRPEASRTGEGSTVFNGAQNGVSQLIQREFQTSAISRDIDTAAKFIGAGAATVGVAGSGAGIGTVFGSLIIGYARNPSLKQQLFSYAILGFALSEAMGLFCLMVAFLILFAM

SEQ ID NO: 14 - protein, 72 aa, Listeria ivanovii
MSLGVIAAAIAVGLGALGAGIGNGLIVSKTVEGVARQPEARSMLQSIMFVGVALVEALPIIAVVIAFMVLNK

SEQ ID NO: 15 - protein, 70 aa, Staphylococcus haemolyticus
MGLIAAAIAIGLSALGAGIGNGLIVSRTVEGVARQPEARGQLMSIMFIGIGLVEALPIIGVVIAFMTLFQ

SEQ ID NO: 16 - protein, 70 aa, Staphylococcus lugdunensis
MGLIAAAIAIGLSALGAGIGNGLIVSRTVEGVARQPEARGQLMSIMFIGIGLVEALPIIGVVIAFMTLFR

SEQ ID NO: 17 - protein, 70 aa, Staphylococcus epidermidis; identical to SEQ ID NO: 5

SEQ ID NO: 18 - protein, 70 aa, Staphylococcus pasteuri; identical to SEQ ID NO: 5

SEQ ID NO: 19 - protein, 70 aa, Staphylococcus warneri; identical to SEQ ID NO: 5

SEQ ID NO: 20 - protein, 68 aa, Staphylococcus saprophyticus
MNLIAAAIAIGLSALGAGIGNGLIVSRTVEGVARQPEARGQLMGIMFIGIGLVEALPIIGVVIAFMSL

SEQ ID NO: 21 - protein, 72 aa, Bacillus coagulans
MSLGILAAAIAVGLAALGAGIGNGLIVGRTVEGIARQPEARGLLQTTMFIGIGLVEALPIIAVVIAFIALGR

SEQ ID NO: 22 - protein, 72 aa, Artificial sequence
  Synthetic sequence
  misc_feature (2)..(2): Xaa can be any naturally occurring amino acid
  misc_feature (4)..(6): Xaa can be any naturally occurring amino acid
  misc_feature (12)..(12): Xaa can be any naturally occurring amino acid
  misc_feature (15)..(15): Xaa can be any naturally occurring amino acid
  misc_feature (28)..(29): Xaa can be any naturally occurring amino acid
  misc_feature (31)..(31): Xaa can be any naturally occurring amino acid
  misc_feature (34)..(34): Xaa can be any naturally occurring amino acid
  misc_feature (40)..(43): Xaa can be any naturally occurring amino acid
  misc_feature (45)..(47): Xaa can be any naturally occurring amino acid
  misc_feature (50)..(50): Xaa can be any naturally occurring amino acid
  misc_feature (52)..(53): Xaa can be any naturally occurring amino acid
  misc_feature (62)..(62): Xaa can be any naturally occurring amino acid
  misc_feature (68)..(72): Xaa can be any naturally occurring amino acid
MXLXXXAAAIAXGLXALGAGIGNGLIVXXTXEGXARQPEXXXXLXXXMFXGXXLVEALPIIXVVIAFXXXXX

SEQ ID NO: 23 - protein, 72 aa, Artificial sequence
  Synthetic sequence
  misc_feature (2)..(2): Xaa can be any naturally occurring amino acid
  misc_feature (4)..(5): Xaa can be any naturally occurring amino acid
  misc_feature (12)..(12): Xaa can be any naturally occurring amino acid
  misc_feature (15)..(15): Xaa can be any naturally occurring amino acid
  misc_feature (29)..(29): Xaa can be any naturally occurring amino acid
  misc_feature (31)..(31): Xaa can be any naturally occurring amino acid
  misc_feature (34)..(34): Xaa can be any naturally occurring amino acid
  misc_feature (40)..(43): Xaa can be any naturally occurring amino acid
  misc_feature (45)..(47): Xaa can be any naturally occurring amino acid
  misc_feature (50)..(50): Xaa can be any naturally occurring amino acid
  misc_feature (52)..(53): Xaa can be any naturally occurring amino acid
  misc_feature (62)..(62): Xaa can be any naturally occurring amino acid
  misc_feature (68)..(72): Xaa can be any naturally occurring amino acid
MXLXXIAAAIAXGLXALGAGIGNGLIVSXTXEGXARQPEXXXXLXXXMFXGXXLVEALPIIXVVIAFXXXXX

SEQ ID NO: 24 - protein, 38 aa, Artificial sequence
  Synthetic sequence
  misc_feature (2)..(4): Xaa can be any naturally occurring amino acid
  misc_feature (10)..(10): Xaa can be any naturally occurring amino acid
  misc_feature (13)..(13): Xaa can be any naturally occurring amino acid
  misc_feature (26)..(27): Xaa can be any naturally occurring amino acid
  misc_feature (29)..(29): Xaa can be any naturally occurring amino acid
  misc_feature (32)..(32): Xaa can be any naturally occurring amino acid
  misc_feature (38)..(38): Xaa can be any naturally occurring amino acid
LXXXAAAIAXGLXALGAGIGNGLIVXXTXEGXARQPEX

SEQ ID NO: 25 - protein, 38 aa, Artificial sequence; identical to SEQ ID NO: 24
  Synthetic sequence
  misc_feature (2)..(3): Xaa is any aliphatic amino acid residue or absent
  misc_feature (4)..(4): Xaa is any aliphatic amino acid residue
  misc_feature (10)..(10): Xaa is any aliphatic amino acid residue
  misc_feature (13)..(13): Xaa is any aliphatic or hydroxyl- or sulfur-containing amino acid residue
  misc_feature (26)..(26): Xaa is any aliphatic or hydroxyl- or sulfur-containing amino acid residue
  misc_feature (27)..(27): Xaa is any basic amino acid residue
  misc_feature (29)..(29): Xaa is any aliphatic amino acid residue
  misc_feature (32)..(32): Xaa is any aliphatic amino acid residue
  MISC_FEATURE (38)..(38): Xaa is any aliphatic amino acid residue

SEQ ID NO: 26 - protein, 38 aa, Artificial sequence; identical to SEQ ID NO: 24
  Synthetic sequence
  misc_feature (2)..(2): Xaa is glycine or absent
  misc_feature (3)..(3): Xaa is valine or absent
  misc_feature (4)..(4): Xaa is isoleucine or leucine
  misc_feature (10)..(10): Xaa is valine or isoleucine
  misc_feature (13)..(13): Xaa is glycine, serine or alanine
  misc_feature (26)..(26): Xaa is serine or glycine
  misc_feature (27)..(27): Xaa is lysine or arginine
  misc_feature (29)..(29): Xaa is valine or isoleucine
  misc_feature (32)..(32): Xaa is valine or isoleucine
  misc_feature (38)..(38): Xaa is alanine or leucine

SEQ ID NO: 27 - protein, 38 aa, Artificial sequence
  Synthetic sequence
  misc_feature (2)..(3): Xaa can be any naturally occurring amino acid
  misc_feature (10)..(10): Xaa can be any naturally occurring amino acid
  misc_feature (13)..(13): Xaa can be any naturally occurring amino acid
  misc_feature (27)..(27): Xaa can be any naturally occurring amino acid
  misc_feature (29)..(29): Xaa can be any naturally occurring amino acid
  misc_feature (32)..(32): Xaa can be any naturally occurring amino acid
  misc_feature (38)..(38): Xaa can be any naturally occurring amino acid
LXXIAAAIAXGLXALGAGIGNGLIVSXTXEGXARQPEX

SEQ ID NO: 28 - protein, 38 aa, Artificial sequence; identical to SEQ ID NO: 27
  Synthetic sequence
  misc_feature (2)..(3): Xaa is any aliphatic amino acid residue or absent
  misc_feature (10)..(10): Xaa is any aliphatic amino acid residue
  misc_feature (13)..(13): Xaa is any aliphatic or hydroxyl- or sulfur-containing amino acid residue
  misc_feature (27)..(27): Xaa is any basic amino acid residue
  misc_feature (29)..(29): Xaa is any aliphatic amino acid residue
  misc_feature (32)..(32): Xaa is any aliphatic amino acid residue
  misc_feature (38)..(38): Xaa is any aliphatic amino acid residue

SEQ ID NO: 29 - protein, 38 aa, Artificial sequence; identical to SEQ ID NO: 27
  Synthetic sequence
  misc_feature (2)..(2): Xaa is glycine or absent
  misc_feature (3)..(3): Xaa is valine or absent
  misc_feature (10)..(10): Xaa is valine or isoleucine
  misc_feature (13)..(13): Xaa is glycine or serine
  misc_feature (27)..(27): Xaa is lysine or arginine
  misc_feature (29)..(29): Xaa is valine or isoleucine
  misc_feature (32)..(32): Xaa is valine or isoleucine
  misc_feature (38)..(38): Xaa is alanine or leucine

SEQ ID NO: 30 - protein, 17 aa, Artificial sequence
  Synthetic sequence
  misc_feature (2)..(3): Xaa can be any naturally occurring amino acid
  misc_feature (12)..(12): Xaa can be any naturally occurring amino acid
GXXLVEALPIIXVVIAF

SEQ ID NO: 31 - protein, 17 aa, Artificial sequence
  Synthetic sequence
  misc_feature (2)..(3): Xaa is any aliphatic amino acid residue
  misc_feature (12)..(12): Xaa is any aliphatic amino acid residue
GXXLVEALPIIXVVIAF

SEQ ID NO: 32 - protein, 17 aa, Artificial sequence
  Synthetic sequence
  misc_feature (2)..(2): Xaa is valine or isoleucine
  misc_feature (3)..(3): Xaa is glycine or alanine
  misc_feature (12)..(12): Xaa is glycine or alanine
GXXLVEALPIIXVVIAF

SEQ ID NO: 33 - protein, 7 aa, Artificial sequence
  Synthetic sequence
ALGAGIG

SEQ ID NO: 34 - protein, 5 aa, Artificial sequence
  Synthetic sequence
LGAGI

SEQ ID NO: 35 - protein, 5 aa, Artificial sequence
  Synthetic sequence
ALGAG

SEQ ID NO: 36 - protein, 5 aa, Artificial sequence
  Synthetic sequence
GAGIG